European Patent Application EP 4 527 417 A1, published March 26, 2025. Title: 抗腫瘍剤及びその利用. Applicant: G F Mille Co., Ltd. The sequence listing filed with the application follows.

SEQUENCE LISTING (11 sequences)

SEQ ID NO: 1 - RNA, 1502 nt, Homo sapiens
  source 1..1502: mol_type = mRNA
accaaacctcttcgaggcacaaggcacaacaggctgctctgggattctcttcagccaatcttcattgctcaagtgtctgaagcagccatggcagaagtacctgagctcgccagtgaaatgatggcttattacagtggcaatgaggatgacttgttctttgaagctgatggccctaaacagatgaagtgctccttccaggacctggacctctgccctctggatggcggcatccagctacgaatctccgaccaccactacagcaagggcttcaggcaggccgcgtcagttgttgtggccatggacaagctgaggaagatgctggttccctgcccacagaccttccaggagaatgacctgagcaccttctttcccttcatctttgaagaagaacctatcttcttcgacacatgggataacgaggcttatgtgcacgatgcacctgtacgatcactgaactgcacgctccgggactcacagcaaaaaagcttggtgatgtctggtccatatgaactgaaagctctccacctccagggacaggatatggagcaacaagtggtgttctccatgtcctttgtacaaggagaagaaagtaatgacaaaatacctgtggccttgggcctcaaggaaaagaatctgtacctgtcctgcgtgttgaaagatgataagcccactctacagctggagagtgtagatcccaaaaattacccaaagaagaagatggaaaagcgatttgtcttcaacaagatagaaatcaataacaagctggaatttgagtctgcccagttccccaactggtacatcagcacctctcaagcagaaaacatgcccgtcttcctgggagggaccaaaggcggccaggatataactgacttcaccatgcaatttgtgtcttcctaaagagagctgtacccagagagtcctgtgctgaatgtggactcaatccctagggctggcagaaagggaacagaaaggtttttgagtacggctatagcctggactttcctgttgtctacaccaatgcccaactgcctgccttagggtagtgctaagaggatctcctgtccatcagccaggacagtcagctctctcctttcagggccaatccccagcccttttgttgagccaggcctctctcacctctcctactcacttaaagcccgcctgacagaaaccacggccacatttggttctaagaaaccctctgtcattcgctcccacattctgatgagcaaccgcttccctatttatttatttatttgtttgtttgttttattcattggtctaatttattcaaagggggcaagaagtagcagtgtctgtaaaagagcctagtttttaatagctatggaatcaattcaatttggactggtgtgctctctttaaatcaagtcctttaattaagactgaaaatatataagctcagattatttaaatgggaatatttataaatgagcaaatatcatactgttcaatggttctgaaataaacttcactgaagaaaa

SEQ ID NO: 2 - RNA, 605 nt, Homo sapiens
  source 1..605: mol_type = mRNA
agagagctgtacccagagagtcctgtgctgaatgtggactcaatccctagggctggcagaaagggaacagaaaggtttttgagtacggctatagcctggactttcctgttgtctacaccaatgcccaactgcctgccttagggtagtgctaagaggatctcctgtccatcagccaggacagtcagctctctcctttcagggccaatccccagcccttttgttgagccaggcctctctcacctctcctactcacttaaagcccgcctgacagaaaccacggccacatttggttctaagaaaccctctgtcattcgctcccacattctgatgagcaaccgcttccctatttatttatttatttgtttgtttgttttattcattggtctaatttattcaaagggggcaagaagtagcagtgtctgtaaaagagcctagtttttaatagctatggaatcaattcaatttggactggtgtgctctctttaaatcaagtcctttaattaagactgaaaatatataagctcagattatttaaatgggaatatttataaatgagcaaatatcatactgttcaatggttctgaaataaacttcactgaagaaaa

SEQ ID NO: 3 - RNA, 1502 nt, Homo sapiens
  source 1..1502: mol_type = mRNA
accaaacctcttcgaggcacaaggcacaacaggctgctctgggattctcttcagccaatcttcattgctcaagtgtctgaagcagccatggcagaagtacctgagctcgccagtgaaatgatggcttattacagtggcaatgaggatgacttgttctttgaagctgatggccctaaacagatgaagtgctccttctaggacctggacctctgccctctggatggcggcatccagctacgaatctccgaccaccactacagcaagggcttcaggcaggccgcgtcagttgttgtggccatggacaagctgaggaagatgctggttccctgcccacagaccttccaggagaatgacctgagcaccttctttcccttcatctttgaagaagaacctatcttcttcgacacatgagataacgaggcttatgtgcacgatgcacctgtacgatcactgaactgcacgctccgggactcacagcaaaaaagcttggtgatgtctggtccatatgaactgaaagctctccacctccagggacaggatatggagcaacaagtggtgttctccatgtcctttgtacaaggagaagaaagtaatgacaaaatacctgtggccttgggcctcaaggaaaagaatctgtacctgtcctgagtgttgaaagatgataagcccactctacagctggagagtgtagatcccaaaaattacccaaagaagaagatggaaaagcgatttgtcttcaacaagatagaaatcaataacaagctggaatttgagtctgcccagttccccaactggtacatcagcacctctcaagcagaaaacatgcccgtcttcctgggagggaccaaaggcggccaggatataactgacttcaccatgcaatttgtgtcttcctaaagagagctgtacccagagagtcctgtgctgaatgtggactcaatccctagggctggcagaaagggaacagaaaggtttttgagtacggctatagcctggactttcctgttgtctacaccaatgcccaactgcctgccttagggtagtgctaagaggatctcctgtccatcagccaggacagtcagctctctcctttcagggccaatccccagcccttttgttgagccaggcctctctcacctctcctactcacttaaagcccgcctgacagaaaccacggccacatttggttctaagaaaccctctgtcattcgctcccacattctgatgagcaaccgcttccctatttatttatttatttgtttgtttgttttattcattggtctaatttattcaaagggggcaagaagtagcagtgtctgtaaaagagcctagtttttaatagctatggaatcaattcaatttggactggtgtgctctctttaaatcaagtcctttaattaagactgaaaatatataagctcagattatttaaatgggaatatttataaatgagcaaatatcatactgttcaatggttctgaaataaacttcactgaagaaaa

SEQ ID NO: 4 - RNA, 130 nt, Homo sapiens
  source 1..130: mol_type = mRNA
ctgtcattcgctcccacattctgatgagcaaccgcttccctatttatttatttatttgtttgtttgttttattcattggtctaatttattcaaaggggacaagaagtagcagtgtctgtaaaagagccta

SEQ ID NO: 5 - RNA, 150 nt, Homo sapiens
  source 1..150: mol_type = mRNA
atttatttatttatttgtttgtttgttttattcattggtctaatttattcaaagggggcaagaagtagcagtgtctgtaaaagagcctagtttttaatagctatggaatcaattcaatttggactggtgtgctctctttaaatcaagtcc

SEQ ID NO: 6 - RNA, 50 nt, Homo sapiens
  source 1..50: mol_type = mRNA
cctatttatttatttatttgtttgtttgttttattcattggtctaattta

SEQ ID NO: 7 - DNA, 28 bp, synthetic construct
  misc_feature 1..28: note = Primer
  source 1..28: mol_type = other DNA
ggtaccatggagcatcggagcaagatgg

SEQ ID NO: 8 - DNA, 30 bp, synthetic construct
  misc_feature 1..30: note = Primer
  source 1..30: mol_type = other DNA
ctcgagttaaggatcccccaacggagcacc

SEQ ID NO: 9 - RNA, 50 nt, synthetic construct
  misc_feature 1..50: note = Control
  source 1..50: mol_type = other RNA
acaaaaaaaaaaaaaaaaaaaaaaaaaaaaaaaaaaaaaaaaaaaaaaca

SEQ ID NO: 10 - RNA, 50 nt, Homo sapiens
  source 1..50: mol_type = mRNA
tatttatttatttatttgtttgtttgttttattcattggtctaatttatt

SEQ ID NO: 11 - RNA, 50 nt, Mus musculus
  source 1..50: mol_type = mRNA
tatttatttatgtatttattgattggttgatctatttaagttgattcaat